European Patent Specification EP 3 708 577 B1, published September 4, 2024. Title: TREATMENT OF BILIARY CIRRHOSIS BASED ON OXYNTOMODULIN ANALOGUE GLP-1R/GCGR DUAL TARGET AGONIST POLYPEPTIDE. Applicant: Shenzhen Turier Biotech Co., Ltd. The sequence listing filed with the application follows.

SEQUENCE LISTING (48 sequences)

SEQ ID NO: 1 - protein, 40 aa, Artificial
  Compound 1
  MISC_FEATURE (2)..(2): D-Ser
  MISC_FEATURE (16)..(16): X=Aib
HSQGTFTSDYSKKLDXRRAQDFVQWLMNTGGPSSGAPPPS

SEQ ID NO: 2 - protein, 40 aa, Artificial; identical to SEQ ID NO: 1
  Compound 2
  MISC_FEATURE (2)..(2): D-Ser
  MISC_FEATURE (16)..(16): X=Aib

SEQ ID NO: 3 - protein, 40 aa, Artificial; identical to SEQ ID NO: 1
  Compound 3
  MISC_FEATURE (2)..(2): D-Ser
  MISC_FEATURE (16)..(16): X=Aib

SEQ ID NO: 4 - protein, 40 aa, Artificial
  Compound 4
  MISC_FEATURE (2)..(2): D-Ser
  MISC_FEATURE (16)..(16): X=Aib
HSQGTFTSDKSKYLDXRRAQDFVQWLMNTGGPSSGAPPPS

SEQ ID NO: 5 - protein, 40 aa, Artificial; identical to SEQ ID NO: 4
  Compound 5
  MISC_FEATURE (2)..(2): D-Ser
  MISC_FEATURE (16)..(16): X=Aib

SEQ ID NO: 6 - protein, 40 aa, Artificial
  Compound 6
  MISC_FEATURE (2)..(2): D-Ser
HSQGTFTSDYSKYLDKRRAQDFVQWLMNTGGPSSGAPPPS

SEQ ID NO: 7 - protein, 40 aa, Artificial
  Compound 7
  MISC_FEATURE (2)..(2): D-Ser
  MISC_FEATURE (16)..(16): X=Aib
HSQGTFTSDYSKYLDXKRAQDFVQWLMNTGGPSSGAPPPS

SEQ ID NO: 8 - protein, 39 aa, Artificial
  Compound 8
  MISC_FEATURE (2)..(2): X=Aib
  MISC_FEATURE (16)..(16): X=Aib
HXQGTFTSDKSKYLDXRRAQDFVQWLLDGGPSSGAPPPS

SEQ ID NO: 9 - protein, 40 aa, Artificial; identical to SEQ ID NO: 1
  Compound 9
  MISC_FEATURE (2)..(2): D-Ser
  MISC_FEATURE (16)..(16): X=Aib

SEQ ID NO: 10 - protein, 40 aa, Artificial; identical to SEQ ID NO: 7
  Compound 10
  MISC_FEATURE (2)..(2): D-Ser
  MISC_FEATURE (16)..(16): X=Aib

SEQ ID NO: 11 - protein, 39 aa, Artificial; identical to SEQ ID NO: 8
  Compound 11
  MISC_FEATURE (2)..(2): X=Aib
  MISC_FEATURE (16)..(16): X=Aib

SEQ ID NO: 12 - protein, 39 aa, Artificial; identical to SEQ ID NO: 8
  Compound 12
  MISC_FEATURE (2)..(2): X=Aib
  MISC_FEATURE (16)..(16): X=Aib

SEQ ID NO: 13 - protein, 39 aa, Artificial
  Compound 13
  MISC_FEATURE (2)..(2): X=Aib
HXQGTFTSDKSKYLDERRAQDFVQWLLDGGPSSGAPPPS

SEQ ID NO: 14 - protein, 39 aa, Artificial; identical to SEQ ID NO: 13
  Compound 14
  MISC_FEATURE (2)..(2): X=Aib

SEQ ID NO: 15 - protein, 39 aa, Artificial; identical to SEQ ID NO: 13
  Compound 15
  MISC_FEATURE (2)..(2): X=Aib

SEQ ID NO: 16 - protein, 39 aa, Artificial; identical to SEQ ID NO: 13
  Compound 16
  MISC_FEATURE (2)..(2): X=Aib

SEQ ID NO: 17 - protein, 29 aa, Artificial
  Compound 17
  MISC_FEATURE (2)..(2): D-Ser
HSQGTFTSDYSKYLDSKAAHDFVEWLLRA

SEQ ID NO: 18 - protein, 29 aa, Artificial
  Compound 18
  MISC_FEATURE (2)..(2): D-Ser
HSQGTFTSDYSKYLDEKAAKEFIEWLLRA

SEQ ID NO: 19 - protein, 39 aa, Artificial; identical to SEQ ID NO: 8
  Compound 19
  MISC_FEATURE (2)..(2): X=Aib
  MISC_FEATURE (16)..(16): X=Aib

SEQ ID NO: 20 - protein, 40 aa, Artificial; identical to SEQ ID NO: 1
  Compound 20
  MISC_FEATURE (2)..(2): D-Ser
  MISC_FEATURE (16)..(16): X=Aib

SEQ ID NO: 21 - protein, 39 aa, Artificial
  Compound 21
  MISC_FEATURE (2)..(2): D-Ser
HSQGTFTSDYSKYLDSKAAHDFVEWLLNGGPSSGAPPPS

SEQ ID NO: 22 - protein, 39 aa, Artificial; identical to SEQ ID NO: 21
  Compound 22
  MISC_FEATURE (2)..(2): D-Ser

SEQ ID NO: 23 - protein, 29 aa, Artificial
  Compound 23
  MISC_FEATURE (2)..(2): D-Ser
HSQGTFTSDYSKYLDEKAAKEFIEWLLRA

SEQ ID NO: 24 - protein, 29 aa, Artificial
  Compound 24
  MISC_FEATURE (2)..(2): D-Ser
HSQGTFTSDYSKYLDEKAAKEFIEWLLRA

SEQ ID NO: 25 - protein, 29 aa, Artificial
  Compound 25
  MISC_FEATURE (2)..(2): D-Ser
HSQGTFTSDYSKYLDSKAAHDFVEWLLRA

SEQ ID NO: 26 - protein, 39 aa, Artificial
  Compound 26
  MISC_FEATURE (2)..(2): D-Ser
HSQGTFTSDYSKYLDEKAAKEFIEWLLNGGPSSGAPPPS

SEQ ID NO: 27 - protein, 39 aa, Artificial; identical to SEQ ID NO: 26
  Compound 27
  MISC_FEATURE (2)..(2): D-Ser

SEQ ID NO: 28 - protein, 39 aa, Artificial; identical to SEQ ID NO: 26
  Compound 28
  MISC_FEATURE (2)..(2): D-Ser

SEQ ID NO: 29 - protein, 39 aa, Artificial; identical to SEQ ID NO: 26
  Compound 29
  MISC_FEATURE (2)..(2): D-Ser

SEQ ID NO: 30 - protein, 40 aa, Artificial; identical to SEQ ID NO: 4
  Compound 30
  MISC_FEATURE (2)..(2): D-Ser
  MISC_FEATURE (16)..(16): X=Aib

SEQ ID NO: 31 - protein, 40 aa, Artificial; identical to SEQ ID NO: 4
  Compound 31
  MISC_FEATURE (2)..(2): D-Ser
  MISC_FEATURE (16)..(16): X=Aib

SEQ ID NO: 32 - protein, 40 aa, Artificial; identical to SEQ ID NO: 4
  Compound 32
  MISC_FEATURE (2)..(2): D-Ser
  MISC_FEATURE (16)..(16): X=Aib

SEQ ID NO: 33 - protein, 40 aa, Artificial; identical to SEQ ID NO: 7
  Compound 33
  MISC_FEATURE (2)..(2): D-Ser
  MISC_FEATURE (16)..(16): X=Aib

SEQ ID NO: 34 - protein, 40 aa, Artificial; identical to SEQ ID NO: 6
  Compound 34
  MISC_FEATURE (2)..(2): D-Ser

SEQ ID NO: 35 - protein, 40 aa, Artificial; identical to SEQ ID NO: 6
  Compound 35
  MISC_FEATURE (2)..(2): D-Ser

SEQ ID NO: 36 - protein, 40 aa, Artificial; identical to SEQ ID NO: 6
  Compound 36
  MISC_FEATURE (2)..(2): D-Ser

SEQ ID NO: 37 - protein, 40 aa, Artificial
  Compound 37
  MISC_FEATURE (2)..(2): D-Ser
  MISC_FEATURE (27)..(27): X=Nle
HSQGTFTSDYSKYLDKRRAQDFVQWLXNTGGPSSGAPPPS

SEQ ID NO: 38 - protein, 40 aa, Artificial; identical to SEQ ID NO: 37
  Compound 38
  MISC_FEATURE (2)..(2): D-Ser
  MISC_FEATURE (27)..(27): X=Nle

SEQ ID NO: 39 - protein, 40 aa, Artificial
  Compound 39
  MISC_FEATURE (2)..(2): D-Ser
HSQGTFTSDYSKYLDKRRAQDFVQWLLNTGGPSSGAPPPS

SEQ ID NO: 40 - protein, 40 aa, Artificial; identical to SEQ ID NO: 39
  Compound 40
  MISC_FEATURE (2)..(2): D-Ser

SEQ ID NO: 41 - protein, 40 aa, Artificial; identical to SEQ ID NO: 37
  Compound 41
  MISC_FEATURE (2)..(2): D-Ser
  MISC_FEATURE (27)..(27): X=Nle

SEQ ID NO: 42 - protein, 40 aa, Artificial; identical to SEQ ID NO: 39
  Compound 42
  MISC_FEATURE (2)..(2): D-Ser

SEQ ID NO: 43 - protein, 40 aa, Artificial
  Compound 43
  MISC_FEATURE (2)..(2): D-Ser
  MISC_FEATURE (16)..(16): X=Aib
HSQGTFTSDKSKYLDXRRAQDFVQWLLNTGGPSSGAPPPS

SEQ ID NO: 44 - protein, 40 aa, Artificial; identical to SEQ ID NO: 43
  Compound 44
  MISC_FEATURE (2)..(2): D-Ser
  MISC_FEATURE (16)..(16): X=Aib

SEQ ID NO: 45 - protein, 40 aa, Artificial
  Compound 45
  MISC_FEATURE (2)..(2): D-Ser
  MISC_FEATURE (16)..(16): X=Aib
  MISC_FEATURE (27)..(27): X=Nle
HSQGTFTSDKSKYLDXRRAQDFVQWLXNTGGPSSGAPPPS

SEQ ID NO: 46 - protein, 40 aa, Artificial; identical to SEQ ID NO: 45
  Compound 46
  MISC_FEATURE (2)..(2): D-Ser
  MISC_FEATURE (16)..(16): X=Aib
  MISC_FEATURE (27)..(27): X=Nle

SEQ ID NO: 47 - protein, 40 aa, Artificial; identical to SEQ ID NO: 43
  Compound 47
  MISC_FEATURE (2)..(2): D-Ser
  MISC_FEATURE (16)..(16): X=Aib

SEQ ID NO: 48 - protein, 40 aa, Artificial; identical to SEQ ID NO: 45
  Compound 48
  MISC_FEATURE (2)..(2): D-Ser
  MISC_FEATURE (16)..(16): X=Aib
  MISC_FEATURE (27)..(27): X=Nle